European Patent Application EP 4 130 265 A1, published February 8, 2023. Title: Method of detecting a single base mutation in erm(41) gene of Mycobacterium abscessus complex, and a probe and a primer set used for the method. Applicant: JAPAN AS REPRESENTED BY DIRECTOR-GENERAL OF NATIONAL INSTITUTE OF INFECTIOUS DISEASES Kaneka Corporation. The sequence listing filed with the application follows.

SEQUENCE LISTING (31 sequences)

SEQ ID NO: 1 - DNA, 522 bp, Mycobacterium abscessus
gtgtccggccaacggtcgcgacgccagtggggctggtatccgctcactgatgactgggcggcgcggatcgtcgccgaatccggtgttcgctcaggggagttcgttgtggatctgggcgcaggacacggcgcgctgacggcacatctggttgccgctggtgccagggtgctagccgtcgagctgcatccggggcgggctcgacaccttcgttcacggtttgccgaggaagatgtccggatagcggaagcggacctgctcgccttccggtggccgcgacggccatttcgggtggtggcgagcccgccctaccaagtcaccagcgcactgatacggagtctcttgacgccggaatcccggctgctggctgccgacctggtgctgcagcgcggggctgtgcacaaacatgcgaagcgagcacctgttcgccattggacgctacgggccggaatcacattgccgcgaagcgctttccatcatccaccgcaggtggattcgtcggtgctggtgatcaggcggcgctga

SEQ ID NO: 2 - DNA, 8336 bp, Mycobacterium abscessus
cgcatacgttagagccattggggcgcattgctttacatcggtttcatactgctgtgttcgtactcgtacgctagtgttcagctgcgtttgtatcaggaaagtggcgacacgggagtcatatctcctttgtcaagctttcgatgatgttgggcaccccggcaccacatgatcgttcgtgatcgagtacaggtaccagttatcggttttgcggagctccacagtggcctcggaggcaaagggttttgggttggggggatctttgagcgtccgccgagtatcagcggtgtaggtgtagcacacgcgcaggaccgctgaaggcggactcagcgcggccagggccgtatcggacaggtgcagatcgtcgtctctgtaaatcctgccctgcgattcgtcagctttctgaactgttccgagttcgtgtaccgcgtcacgcagacggccatattggtctgcctcgagatcgggcaccacgatcttcataaacttggcgtaccgggcgccgccctgatcacaggcaccattgcaagccaccactgcgggccagatgtcgttggcgaaccggggaattaccccgttggtatcgggaacatttgttgacgtgctggcgactggggactgcagaatctccgagggcgcaggcggtggactcgtacatcccgtcagcaccgcaagggttaacgacaggcaggcgagccgggtgcgggtggtcatggcttgagcctgagaacatcggcgctgtcccggcgttccgttacgtcatcaagccttaccgccatgcctgagccgggtgcgttaagcatgaagccgttaccgacgtagagcccggtgtgtggggtacctccaccagtgaacggcgttccgccttcgcggaatacgaggatatcgccgggctgtgcaaagttgtcgatctgcttggacggcacagcttgaggctgaccgtggtcgaagatggggtttatatcgaggcggtcggtccctgggatgtctccgcgtggcacgaacggatcgaaaccggccccttgttgcactgagtaccgcacaagcccgccgcagtcgaacccgatccggttccaatcctcgtaggtatccgctgaggtgcccttttccccatgtccacgtgatggcccgttggggtcggtgttgccgccccaagcgtaggaaactccctgtgagcggccagcggcgccgatcgatcgtaaagccttgtcgctaacagcttctggcttcgggagcgccagcggcggttgacctgccgcgcgctgtgtgccgtcggcattcttgccggataggtagtctttccaggcttgatcacgtgctggtcccgggccggtgttctggtcgtagcctggcggattgtccgccatgggaatggttttcgcgccatcgatcatcgtgggcttggcaccgttgggatatggcggattaccgtctgcgccgcctacgggctcggaggcattgagcgcgacaggcggggcttgtggtgtaggtgctggtgcgtcggtgacatcggcgcgcagagcggctgcgatttcctgctcaacttgggtggcgcgttgttcgagggtggtgacttgttgttgcaggcgggcgatttggtcgtcttgcaggtgcttgtcagtgtctttgaccttggtcgtggcgacgactttgccgtcgtcggtgatcgtggcgccgattgcttgagcgtcttgatcgagcatgcccagtttgttggtgacctcccgtacgtcatcgatagcgggtttgacggctttagcgaccttctcggcggcatcagccttatcgcccagatctacacgcgtcttgcccgcgctgtctttccacgcccccgcggtgacaccgccccacgtggacagatcattagcgacctgttccataccctccccgaggcgatgcaggctggccgctcgtgctgcggcggtatcgaacagcttctccaacgtctcggctttccaatgccggatatcaccaaccttggccacaatcagctcccgcttcccggcccgccgaaacggccagcgttaccgtcatcggcgccaaccaccttggcggtggcatcaagaatccaagtcgcatgatcgcccacctgtttgcgtatcgcctcgtgctgctggtcccacccggcacgtaagttttccattgctgagccgaccacccctggccagcgagaagctaattcggtcaggtccgcatcgtggccgatgtggtcctggcggtgcgtctccacatggtccaacagcttgttggcctgcctgtgcagcaactccgggtcgaatctcaacggctcggacatatcggcctcccgcccgacttggtgacggccatcaccctgtttgccagcgagcctaacactgcgcccatagtggcgcgatgagacaggtcacccgtgccgttactgccaaggcggcgcgggtggcaccgctcagaacctgcgtgcgctgatggcccagaaccaaaaaggtaggagaatgccgccgtgcgggaggacgaacgtttaggcggcggcttgcaagcgccggctgctggaggcttcccataaggccgctctgggggcctctctcaagaaccgggcatcatttgacctgcgataatgatcaatcggttggtgggtgtcggtcatagccgtcatagtggacgcagatacgatggtgcaatcgaggatctgagaaaggagttccgccgtgaccgtcacagagactgcgtgtgaagtagtggagttgacctcagatgaaggtgccgagttgttcgacagcatcgctcagaacaacatgggcatcacaggggcggagtttgtgcgacgttggaacgcaggggaatttgaagggatcaactgggacgacgttccagggctgacgtcggtcgcgacggcgctgcctttcgcaggcatctgagagacacgtttgccaaagtgcctggtcgcacccctcacgacgcgatccgtaattacatagatccgcttcaacaggcggtttcatgtttagggtgcgccaagatccaactttcacaaacgcccaagaggtacggcgaattcggagcatggatcctcaacgggggcaacggaatggtgctccgaggattcggtaagttctacgccacccagcggtttgagttagttcctacgacagcggatctgcacgatgctcctgaaaaggagccctttcgggtttcgacgcgcgaatatatctaccgactcgaaattgctaatgagagtcatgtcatcgaatggcactggcacccggtagggaacagcgacgagcggcgcccccacatccaccctgcaatcaaccgggatgcgcatctccccggtccccgggtggtgctggaagacgtaatagagggctgtatcgcactaggcgcgacacctgcctgcgaggactggaaagagcggctagccgccagcggtggcgtccacaagctgtacaggacatgggtccacgagcctggcgatctaaagaagcctgcagtaaaagaggactagctagctttcacgtggtcccgaacttgggacgcgtgagcgccaagagccgctgaggccgccgggagagggccacatcgcaccagcagccggtttcaccttccgtggatcgtgttggtggcgaataaaaaacgggatttcagtgacggttgggtgttgaaaacaaattggggcagggggggcgtttgcctaagccatgaggggcgggcgccggacccctcgggttcactcccccggggggtcgtcgtggagtgcggcttgtccgaggcgctcgacgtagccgctgacggtgggcagcactggccgaaatccgcagcgggccacgtgccaggcgtcgcgcagatcagacttgttcttggcgcgggcggcgacgatgcgtgcagcggaggcatcgccgttagggatcaacgtgtgggcgcggtcgccaccgatcccggcagattgcagcagcgcgccgagtccttcgacggcgtagccgaatcgttcgcgcgccacgagggcttcggaccatgcgatgacggctttcggtccggccttggtgatcgtcggcccgtcgttgaggtcatcggtcgggatcacttcagcggcagcttcaagcgaattagcgtatggttcaagggatttagaccactgggccaatatggtgtcggcgtgagcgttgagcgcctcaccgatcgtgcgcccctcctcgtccttggcggcgcggtctaggccgagctgcgcaagcatgtggtcaagaaggtggccggttaccacagggtcagcgtggtaatcctggtccttcttcatgcagctgagcacggagtacctgagggcgtccgcgctgccagcaccgatctgcgccttctcgaccaacgctcgggccgaggccacagcctctacgaatggatcgggcagcggaatttcaaggcgttcggcggcgcgttgcacctggacgaggtaggaacgggttgtggcggtgtagacggacatgtgtttgtctcctagtagttttcgttgaaagcgatttcgccggttagggcttcgcgcaggaagttgatttcgacttgacgcgggtgtttccggggccggtgattgttgccctcgcccggtacgtagttggacgattcaggctgcggtgcgggaggagtgccgaggcgttcgtaaagacgcttaaggtcctcggaatcggcactgtccgttgcggtctcgtcgccacgcagtcgccgtagcagatcggtggcaggggcttcggtgtcactgttgagctgctgtagcacctgcttccagtcgggtttatccatgtggttcttgcctttcgtcgaagatccagcgcccgccgactttgcgttgcccggatttgagtgcgtggcggcggatggtgcggggcgaaactccaaggcgctcagccctttgttgcactgtctccaattctgctcccgccgtttcggggtgtccagaaacctgtccgctatcggacacactgcgctgcaacgcttcccatgttcgatgcaaggccggtgggatcggggtgccttggcggcgacggcgcgctagttcctccccgagcacccatgcggcggtgcgaagatcccgcacgctgaccacgcggtgctctcccgtggcgcattgggtgcaaggctgcgctgtcgtgctcatgccgcccccgtcgcctcgtcctggccgtctttggtggtgatttcctgcttctttcgcggcgggtacgagttgaccaccacggcggcggtaaccccgagcggccgctgctcgtgcggcagggaatcgaaccactcccggcacgaggccagcgcagggcattggcggcatatccgcgtcgctgcctggcgggcgtagtcgcgctcgtccagggcgcctcggccatcgccgatagcggcgtcgaacaactcgtgccgtccccggcagcgcgccccaggcagtacaggcgtggctagttcggccagcagcgtgtcccagttcaccgcgccccctcctggtcctgagcatctgtttcgttgagtgcttgtgcggcagcccaattgccgtgtcgtgggcagtcggtgaggttgtccaggcgcccgtagtcgtcacagtgtgggcagttgcgtatctgccggatcgcttcgcggcgggtgttggcgcgctcgcgtgtcttgcggcagtgtgcgcagtagcggcaggacatcaggcggttctccctccctgggcttgcgcccagctgacgtgacgcgggcagggcttgagtccgtcatcgacttcgatccggcccaagtcgtcgcaatccgggcagtcccgaatcacctgcacggctgcgcgtttgcgttcggcctccgacgccgtggcagccttgcgcagcgctgcgcagtcgcggcagctctcacccacccaggcatcaggtgcgatgtgcgcgtgcttggcgcaacgcgtccccgtctcattgccgttagctgattgccgccctcggctggcgggggtgatcgcgtaggcgtccgggtcgtcaagttccgtacccccataacgcaaccccctcttttgatgtggtcctgatgtggtggggggcaccgccgtgcgggtcaaagaggcaccgccgtacgggctatcggaccgttgacccgcaccgctgtgcgggctttggctgttttgacccgcacggccatgcggggtatcaccgttttgacccgcaccgccatgcggggtatttgcgatcggaaccagccgatacacggcggcatgacgcttgaatccgtttgctgtgcgctggatgagccccagctcgcggcctcgcttgagcgccgtttccacagcccgttcggtgagcccgcatttccgcatgagcccttctattccaggccgcgcgttggtgccgtccgcgtagtcggcgaacgtctcaagcgccaggagaactatccgctgggccaacgtcagggccttggccccgagaacataatcgcgccagtcacggcgctgctctggcgtcacggtaagccgccctgtgcgtcagcaggcaatgcacggcttcggctagcgcgcacgctggcgtgcaactgggccgcgcgatgcacgtcgcagcgcacaacagggcgcacaccatcacgcaccgtgacgcacaactcgtgcactcccccaggcccatcgggcagccgaccaacaagcccgccgcccaatggtgcccgtgcgcactcacgcagaggcatcgcgctccaccgcgtgatgagtgcaatctgttccgatcacaaggactccacgacctcagcggcggcgcgcagcgcatcagtcaggcgtcgcgccgcgctcgcttccatccagtcctcgacaccattgacccaacgcacgccccactcaaccgaaccatctgcggcctgctgggtgccctctatgagcacatgccccaagccctcgcccacctcgaaccgggcgccctctagcctgcgcccccagtccggcgattccttagagcccatgttcatccactggtcagcatgtgaggcttgagctgggatcggcacatgcgcgaaccggataccagcttgatgcgtctcgatatcgagggtgatcttgaaaaggagactcaacgctgcgttgtcggcctgactcgtggcccgccatggcgtgaccccagccgccgccaactcctcggcgcgctccaactgcgctacccagtcagccggtagtcgatcaaccaagtcacgccatgtccgggtgtcgtcgccaaattcgatctgtaccatgagatttacctactttctgttgatggttggttgcagcggctcccgcccgacgttgccgcgtcggggactacgggggccgttggcatagccgaacttgtgccgacgagctgaacttgtgcgcgatattcgcgcttggccccgtcagcgtcggtcacggtcaccgtgatcacatcgccctcggcctccacgctggccgtggaattcggaaccaccttgccatcccgaataatgcatggcgacaagggaacccacggctcttgcgctagccgcgccgcgatcctgtacgcctcgatactcacgccgcgccttcaagcttggcgatgtactcgttgatctgcctgtcagtgctgaatcggcgcttaccaatcctcacgctggcgagggcaccagagtgccagagctggaacaccagcgttctgctgatacctccgagctttgcccccactgccttgtggtcgtgcattgcgtcctcctccgttcatggctgcttgtgcgttcaaacacgcagacatccgataagttgcgtttctgcgactcaatagataccaggcggatggcaatgaacgcaagcagtgcatatcctgcgtgtcatgacgcaatcagggccgaaaaggccgagttggacggaacggccgcccgacagctgggcggaacgtgaagcgcatagattggcgcgcgaggtttaccggcttcgcggaaagaggtcagcgcagtggcttgcggctcggaccaaggaactcggccacgaagtatcccgttcggtgatttccgatttggagaatgggcgacgtaggtatgtcacgaccgctgagctagtaatactcgctgccgcactcgatacgtccccagtaacgctgatgtaccccggcccgtattccgattcggtggaatttctacctgaacgagaagttccggaattcgatgcagcgcagtggttttcggcaaacgggtggtcgcaagagctagcgagtgcgttcgacggcgatttcggatttgcttggcgcacagatcagcttcgccaatggcgacgcctggcggaattggaagatgcccgcgcccgcgtgacggcgcgagccgaacttgaccgtgaccgcgatcaaatcgaaatgtacgacagaatgattcgcgaattgtggcaacaaatcgagggtaacgag

SEQ ID NO: 3 - DNA, 128 bp, Mycobacterium abscessus
cgcatacgttagagccattggggcgcattgctttacatcggtttcatactgctgtgttcgtactcgtacgctagtgttcagctgcgtttgtatcaggaaagtggcgacacgggagtcatatctccttt

SEQ ID NO: 4 - DNA, 2237 bp, Mycobacterium abscessus
gtcaagctttcgatgatgttgggcaccccggcaccacatgatcgttcgtgatcgagtacaggtaccagttatcggttttgcggagctccacagtggcctcggaggcaaagggttttgggttggggggatctttgagcgtccgccgagtatcagcggtgtaggtgtagcacacgcgcaggaccgctgaaggcggactcagcgcggccagggccgtatcggacaggtgcagatcgtcgtctctgtaaatcctgccctgcgattcgtcagctttctgaactgttccgagttcgtgtaccgcgtcacgcagacggccatattggtctgcctcgagatcgggcaccacgatcttcataaacttggcgtaccgggcgccgccctgatcacaggcaccattgcaagccaccactgcgggccagatgtcgttggcgaaccggggaattaccccgttggtatcgggaacatttgttgacgtgctggcgactggggactgcagaatctccgagggcgcaggcggtggactcgtacatcccgtcagcaccgcaagggttaacgacaggcaggcgagccgggtgcgggtggtcatggcttgagcctgagaacatcggcgctgtcccggcgttccgttacgtcatcaagccttaccgccatgcctgagccgggtgcgttaagcatgaagccgttaccgacgtagagcccggtgtgtggggtacctccaccagtgaacggcgttccgccttcgcggaatacgaggatatcgccgggctgtgcaaagttgtcgatctgcttggacggcacagcttgaggctgaccgtggtcgaagatggggtttatatcgaggcggtcggtccctgggatgtctccgcgtggcacgaacggatcgaaaccggccccttgttgcactgagtaccgcacaagcccgccgcagtcgaacccgatccggttccaatcctcgtaggtatccgctgaggtgcccttttccccatgtccacgtgatggcccgttggggtcggtgttgccgccccaagcgtaggaaactccctgtgagcggccagcggcgccgatcgatcgtaaagccttgtcgctaacagcttctggcttcgggagcgccagcggcggttgacctgccgcgcgctgtgtgccgtcggcattcttgccggataggtagtctttccaggcttgatcacgtgctggtcccgggccggtgttctggtcgtagcctggcggattgtccgccatgggaatggttttcgcgccatcgatcatcgtgggcttggcaccgttgggatatggcggattaccgtctgcgccgcctacgggctcggaggcattgagcgcgacaggcggggcttgtggtgtaggtgctggtgcgtcggtgacatcggcgcgcagagcggctgcgatttcctgctcaacttgggtggcgcgttgttcgagggtggtgacttgttgttgcaggcgggcgatttggtcgtcttgcaggtgcttgtcagtgtctttgaccttggtcgtggcgacgactttgccgtcgtcggtgatcgtggcgccgattgcttgagcgtcttgatcgagcatgcccagtttgttggtgacctcccgtacgtcatcgatagcgggtttgacggctttagcgaccttctcggcggcatcagccttatcgcccagatctacacgcgtcttgcccgcgctgtctttccacgcccccgcggtgacaccgccccacgtggacagatcattagcgacctgttccataccctccccgaggcgatgcaggctggccgctcgtgctgcggcggtatcgaacagcttctccaacgtctcggctttccaatgccggatatcaccaaccttggccacaatcagctcccgcttcccggcccgccgaaacggccagcgttaccgtcatcggcgccaaccaccttggcggtggcatcaagaatccaagtcgcatgatcgcccacctgtttgcgtatcgcctcgtgctgctggtcccacccggcacgtaagttttccattgctgagccgaccacccctggccagcgagaagctaattcggtcaggtccgcatcgtggccgatgtggtcctggcggtgcgtctccacatggtccaacagcttgttggcctgcctgtgcagcaactccgggtcgaatctcaacggctcggacatatcggcctcccgcccgacttggtgacggccatcaccctgtttgccagcgagcctaacactgcgcccatagtg

SEQ ID NO: 5 - DNA, 1208 bp, Mycobacterium abscessus
gcgcgatgagacaggtcacccgtgccgttactgccaaggcggcgcgggtggcaccgctcagaacctgcgtgcgctgatggcccagaaccaaaaaggtaggagaatgccgccgtgcgggaggacgaacgtttaggcggcggcttgcaagcgccggctgctggaggcttcccataaggccgctctgggggcctctctcaagaaccgggcatcatttgacctgcgataatgatcaatcggttggtgggtgtcggtcatagccgtcatagtggacgcagatacgatggtgcaatcgaggatctgagaaaggagttccgccgtgaccgtcacagagactgcgtgtgaagtagtggagttgacctcagatgaaggtgccgagttgttcgacagcatcgctcagaacaacatgggcatcacaggggcggagtttgtgcgacgttggaacgcaggggaatttgaagggatcaactgggacgacgttccagggctgacgtcggtcgcgacggcgctgcctttcgcaggcatctgagagacacgtttgccaaagtgcctggtcgcacccctcacgacgcgatccgtaattacatagatccgcttcaacaggcggtttcatgtttagggtgcgccaagatccaactttcacaaacgcccaagaggtacggcgaattcggagcatggatcctcaacgggggcaacggaatggtgctccgaggattcggtaagttctacgccacccagcggtttgagttagttcctacgacagcggatctgcacgatgctcctgaaaaggagccctttcgggtttcgacgcgcgaatatatctaccgactcgaaattgctaatgagagtcatgtcatcgaatggcactggcacccggtagggaacagcgacgagcggcgcccccacatccaccctgcaatcaaccgggatgcgcatctccccggtccccgggtggtgctggaagacgtaatagagggctgtatcgcactaggcgcgacacctgcctgcgaggactggaaagagcggctagccgccagcggtggcgtccacaagctgtacaggacatgggtccacgagcctggcgatctaaagaagcctgcagtaaaagaggactagctagctttcacgtggtcccgaacttgggacgcgtgagcgccaagagccgctgaggccgccgggagagggccacatcgcaccagcagccggtttca

SEQ ID NO: 6 - DNA, 480 bp, Mycobacterium abscessus
ccttccgtggatcgtgttggtggcgaataaaaaacgggatttcagtgacggttgggtgttgaaaacaaattggggcagggggggcgtttgcctaagccatgaggggcgggcgccggacccctcgggttcactcccccggggggtcgtcgtggagtgcggcttgtccgaggcgctcgacgtagccgctgacggtgggcagcactggccgaaatccgcagcgggccacgtgccaggcgtcgcgcagatcagacttgttcttggcgcgggcggcgacgatgcgtgcagcggaggcatcgccgttagggatcaacgtgtgggcgcggtcgccaccgatcccggcagattgcagcagcgcgccgagtccttcgacggcgtagccgaatcgttcgcgcgccacgagggcttcggaccatgcgatgacggctttcggtccggccttggtgatcgtcggcccgtcgttgaggtcatcggtcgggatca

SEQ ID NO: 7 - DNA, 1040 bp, Mycobacterium abscessus
cttcagcggcagcttcaagcgaattagcgtatggttcaagggatttagaccactgggccaatatggtgtcggcgtgagcgttgagcgcctcaccgatcgtgcgcccctcctcgtccttggcggcgcggtctaggccgagctgcgcaagcatgtggtcaagaaggtggccggttaccacagggtcagcgtggtaatcctggtccttcttcatgcagctgagcacggagtacctgagggcgtccgcgctgccagcaccgatctgcgccttctcgaccaacgctcgggccgaggccacagcctctacgaatggatcgggcagcggaatttcaaggcgttcggcggcgcgttgcacctggacgaggtaggaacgggttgtggcggtgtagacggacatgtgtttgtctcctagtagttttcgttgaaagcgatttcgccggttagggcttcgcgcaggaagttgatttcgacttgacgcgggtgtttccggggccggtgattgttgccctcgcccggtacgtagttggacgattcaggctgcggtgcgggaggagtgccgaggcgttcgtaaagacgcttaaggtcctcggaatcggcactgtccgttgcggtctcgtcgccacgcagtcgccgtagcagatcggtggcaggggcttcggtgtcactgttgagctgctgtagcacctgcttccagtcgggtttatccatgtggttcttgcctttcgtcgaagatccagcgcccgccgactttgcgttgcccggatttgagtgcgtggcggcggatggtgcggggcgaaactccaaggcgctcagccctttgttgcactgtctccaattctgctcccgccgtttcggggtgtccagaaacctgtccgctatcggacacactgcgctgcaacgcttcccatgttcgatgcaaggccggtgggatcggggtgccttggcggcgacggcgcgctagttcctccccgagcacccatgcggcggtgcgaagatcccgcacgctgaccacgcggtgctctcccgtggcgcattgggtgcaa

SEQ ID NO: 8 - DNA, 1338 bp, Mycobacterium abscessus
ggctgcgctgtcgtgctcatgccgcccccgtcgcctcgtcctggccgtctttggtggtgatttcctgcttctttcgcggcgggtacgagttgaccaccacggcggcggtaaccccgagcggccgctgctcgtgcggcagggaatcgaaccactcccggcacgaggccagcgcagggcattggcggcatatccgcgtcgctgcctggcgggcgtagtcgcgctcgtccagggcgcctcggccatcgccgatagcggcgtcgaacaactcgtgccgtccccggcagcgcgccccaggcagtacaggcgtggctagttcggccagcagcgtgtcccagttcaccgcgccccctcctggtcctgagcatctgtttcgttgagtgcttgtgcggcagcccaattgccgtgtcgtgggcagtcggtgaggttgtccaggcgcccgtagtcgtcacagtgtgggcagttgcgtatctgccggatcgcttcgcggcgggtgttggcgcgctcgcgtgtcttgcggcagtgtgcgcagtagcggcaggacatcaggcggttctccctccctgggcttgcgcccagctgacgtgacgcgggcagggcttgagtccgtcatcgacttcgatccggcccaagtcgtcgcaatccgggcagtcccgaatcacctgcacggctgcgcgtttgcgttcggcctccgacgccgtggcagccttgcgcagcgctgcgcagtcgcggcagctctcacccacccaggcatcaggtgcgatgtgcgcgtgcttggcgcaacgcgtccccgtctcattgccgttagctgattgccgccctcggctggcgggggtgatcgcgtaggcgtccgggtcgtcaagttccgtacccccataacgcaaccccctcttttgatgtggtcctgatgtggtggggggcaccgccgtgcgggtcaaagaggcaccgccgtacgggctatcggaccgttgacccgcaccgctgtgcgggctttggctgttttgacccgcacggccatgcggggtatcaccgttttgacccgcaccgccatgcggggtatttgcgatcggaaccagccgatacacggcggcatgacgcttgaatccgtttgctgtgcgctggatgagccccagctcgcggcctcgcttgagcgccgtttccacagcccgttcggtgagcccgcatttccgcatgagcccttctattccaggccgcgcgttggtgccgtccgcgtagtcggcgaacgtctcaagcgccaggagaactatccgctgggccaacgtcagggccttggccccgagaacataatcgcgccagtcacggcgctgctctggcgtcacg

SEQ ID NO: 9 - DNA, 164 bp, Mycobacterium abscessus
gtaagccgccctgtgcgtcagcaggcaatgcacggcttcggctagcgcgcacgctggcgtgcaactgggccgcgcgatgcacgtcgcagcgcacaacagggcgcacaccatcacgcaccgtgacgcacaactcgtgcactcccccaggcccatcgggcagccga

SEQ ID NO: 10 - DNA, 892 bp, Mycobacterium abscessus
ccaacaagcccgccgcccaatggtgcccgtgcgcactcacgcagaggcatcgcgctccaccgcgtgatgagtgcaatctgttccgatcacaaggactccacgacctcagcggcggcgcgcagcgcatcagtcaggcgtcgcgccgcgctcgcttccatccagtcctcgacaccattgacccaacgcacgccccactcaaccgaaccatctgcggcctgctgggtgccctctatgagcacatgccccaagccctcgcccacctcgaaccgggcgccctctagcctgcgcccccagtccggcgattccttagagcccatgttcatccactggtcagcatgtgaggcttgagctgggatcggcacatgcgcgaaccggataccagcttgatgcgtctcgatatcgagggtgatcttgaaaaggagactcaacgctgcgttgtcggcctgactcgtggcccgccatggcgtgaccccagccgccgccaactcctcggcgcgctccaactgcgctacccagtcagccggtagtcgatcaaccaagtcacgccatgtccgggtgtcgtcgccaaattcgatctgtaccatgagatttacctactttctgttgatggttggttgcagcggctcccgcccgacgttgccgcgtcggggactacgggggccgttggcatagccgaacttgtgccgacgagctgaacttgtgcgcgatattcgcgcttggccccgtcagcgtcggtcacggtcaccgtgatcacatcgccctcggcctccacgctggccgtggaattcggaaccaccttgccatcccgaataatgcatggcgacaagggaacccacggctcttgcgctagccgcgccgcgatcctgtacgcctcgatactcacgccgcgcct

SEQ ID NO: 11 - DNA, 849 bp, Mycobacterium abscessus
tcaagcttggcgatgtactcgttgatctgcctgtcagtgctgaatcggcgcttaccaatcctcacgctggcgagggcaccagagtgccagagctggaacaccagcgttctgctgatacctccgagctttgcccccactgccttgtggtcgtgcattgcgtcctcctccgttcatggctgcttgtgcgttcaaacacgcagacatccgataagttgcgtttctgcgactcaatagataccaggcggatggcaatgaacgcaagcagtgcatatcctgcgtgtcatgacgcaatcagggccgaaaaggccgagttggacggaacggccgcccgacagctgggcggaacgtgaagcgcatagattggcgcgcgaggtttaccggcttcgcggaaagaggtcagcgcagtggcttgcggctcggaccaaggaactcggccacgaagtatcccgttcggtgatttccgatttggagaatgggcgacgtaggtatgtcacgaccgctgagctagtaatactcgctgccgcactcgatacgtccccagtaacgctgatgtaccccggcccgtattccgattcggtggaatttctacctgaacgagaagttccggaattcgatgcagcgcagtggttttcggcaaacgggtggtcgcaagagctagcgagtgcgttcgacggcgatttcggatttgcttggcgcacagatcagcttcgccaatggcgacgcctggcggaattggaagatgcccgcgcccgcgtgacggcgcgagccgaacttgaccgtgaccgcgatcaaatcgaaatgtacgacagaatgattcgcgaattgtggcaacaaatcgagggtaacgag

SEQ ID NO: 12 - DNA, 25 bp, Artificial
  C28-f primer
tcctcggaatcggcactgtccgttg

SEQ ID NO: 13 - DNA, 27 bp, Artificial
  C28-r primer
tacagcagctcaacagtgacaccgaag

SEQ ID NO: 14 - DNA, 27 bp, Artificial
  tag
tggcaacatttttcactgggtttatag

SEQ ID NO: 15 - DNA, 27 bp, Artificial
  tag
tgcatcgagtgacagctaatgtgtgat

SEQ ID NO: 16 - DNA, 27 bp, Artificial
  tag
ctataaacccagtgaaaaatgttgcca

SEQ ID NO: 17 - DNA, 27 bp, Artificial
  tag
atcacacattagctgtcactcgatgca

SEQ ID NO: 18 - DNA, 22 bp, Artificial
  1-C28-1f primer
gcgcgatgagacaggtcacccg

SEQ ID NO: 19 - DNA, 20 bp, Artificial
  1-C28-1r primer
gcagtctctgtgacggtcac

SEQ ID NO: 20 - DNA, 20 bp, Artificial
  1-C28-2f primer
gacgcagatacgatggtgca

SEQ ID NO: 21 - DNA, 25 bp, Artificial
  1-C28-2r primer
tgaaaccggctgctggtgcgatgtg

SEQ ID NO: 22 - DNA, 20 bp, Artificial
  2-C28-1f primer
cttcagcggcagcttcaagc

SEQ ID NO: 23 - DNA, 23 bp, Artificial
  2-C28-1r primer
ttgcacccaatgcgccacgggag

SEQ ID NO: 24 - DNA, 21 bp, Artificial
  3-C28-1f primer
cgcaccgtgacgcacaactcg

SEQ ID NO: 25 - DNA, 20 bp, Artificial
  3-C28-1r primer
tcggctgcccgatgggcctg

SEQ ID NO: 26 - DNA, 23 bp, Artificial
  4-C28-1f primer
tcaagcttggcgatgtactcgtt

SEQ ID NO: 27 - DNA, 26 bp, Artificial
  4-C28-1r primer
cgcccattctccaaatcggaaatcac

SEQ ID NO: 28 - DNA, 25 bp, Artificial
  4-C28-2f primer
gcattgcgtcctcctccgttcatgg

SEQ ID NO: 29 - DNA, 25 bp, Artificial
  4-C28-2r primer
ctcgttaccctcgatttgttgccac

SEQ ID NO: 30 - DNA, 17 bp, Artificial
  T28-1f primer
gatgagtgcgcccgaag

SEQ ID NO: 31 - DNA, 18 bp, Artificial
  T28-1r primer
tctactcgtcgccgcttg